European Patent Application EP 4 342 498 A1, published March 27, 2024. Title: Antisense Oligomer. Applicant: NATIONAL UNIVERSITY CORPORATION CHIBA UNIVERSITY. The sequence listing filed with the application follows.

SEQUENCE LISTING (41 sequences)

SEQ ID NO: 1 - DNA, 116 bp, Homo sapiens
ttaattttattattttttagttcgaaaactgtatcttcgggcaccaaagagcattgttataatcaagtaccagttgaattaagtacagagaagaaggtttgttttaaagaaattgt

SEQ ID NO: 2 - DNA, 9 bp, Homo sapiens
gttcgaaaa

SEQ ID NO: 3 - DNA, 9 bp, Homo sapiens
agaagaagg

SEQ ID NO: 4 - DNA, 21 bp, Homo sapiens
ttagttcgaaaactgtatctt

SEQ ID NO: 5 - DNA, 21 bp, Homo sapiens
taagtacagagaagaaggttt

SEQ ID NO: 6 - DNA, 30 bp, Homo sapiens
ttttttagttcgaaaactgtatcttcgggc

SEQ ID NO: 7 - DNA, 30 bp, Homo sapiens
tttttagttcgaaaactgtatcttcgggca

SEQ ID NO: 8 - DNA, 30 bp, Homo sapiens
ttttagttcgaaaactgtatcttcgggcac

SEQ ID NO: 9 - DNA, 30 bp, Homo sapiens
tttagttcgaaaactgtatcttcgggcacc

SEQ ID NO: 10 - DNA, 30 bp, Homo sapiens
ttagttcgaaaactgtatcttcgggcacca

SEQ ID NO: 11 - DNA, 30 bp, Homo sapiens
tgaattaagtacagagaagaaggtttgttt

SEQ ID NO: 12 - DNA, 30 bp, Homo sapiens
ttgaattaagtacagagaagaaggtttgtt

SEQ ID NO: 13 - DNA, 30 bp, Homo sapiens
gttgaattaagtacagagaagaaggtttgt

SEQ ID NO: 14 - DNA, 30 bp, Homo sapiens
agttgaattaagtacagagaagaaggtttg

SEQ ID NO: 15 - DNA, 30 bp, Homo sapiens
cagttgaattaagtacagagaagaaggttt

SEQ ID NO: 16 - DNA, 78 bp, Homo sapiens
gttcgaaaactgtatcttcgggcaccaaagagcattgttataatcaagtaccagttgaattaagtacagagaagaagg

SEQ ID NO: 17 - DNA, 25 bp, Artificial Sequence
  Synthetic antisense oligomer
cgaagatacagttttcgaactaaaa

SEQ ID NO: 18 - DNA, 25 bp, Artificial Sequence
  Synthetic antisense oligomer
acaaaccttcttctctgtacttaat

SEQ ID NO: 19 - DNA, 30 bp, Artificial Sequence
  Synthetic antisense oligomer
acaaaccttcttctctgtacttaattcaac

SEQ ID NO: 20 - DNA, 25 bp, Artificial Sequence
  Synthetic antisense oligomer
cctcttacctcagttacaatttata

SEQ ID NO: 21 - DNA, 105 bp, Artificial Sequence
  Synthetic DNA oligomer
ccggtaaaacaaaccttcttctctgtacttaattcaactggtacttgattataacaatgctctttggtgcccgaagatacagtcttcgaactaaaaaatattttt

SEQ ID NO: 22 - DNA, 105 bp, Artificial Sequence
  Synthetic DNA oligomer
aattaaaaatattttttagttcgaagactgtatcttcgggcaccaaagagcattgttataatcaagtaccagttgaattaagtacagagaagaaggtttgtttta

SEQ ID NO: 23 - DNA, 20 bp, Artificial Sequence
  Synthetic DNA oligomer
tggcactggcaaggatcaaa

SEQ ID NO: 24 - DNA, 25 bp, Artificial Sequence
  Synthetic DNA oligomer
tcccagaagaaatcttatcacatgg

SEQ ID NO: 25 - DNA, 30 bp, Artificial sequence
  Synthetic antisense oligomer
gcccgaagatacagttttcgaactaaaaaa

SEQ ID NO: 26 - DNA, 30 bp, Artificial sequence
  Synthetic antisense oligomer
tgcccgaagatacagttttcgaactaaaaa

SEQ ID NO: 27 - DNA, 30 bp, Artificial sequence
  Synthetic antisense oligomer
gtgcccgaagatacagttttcgaactaaaa

SEQ ID NO: 28 - DNA, 30 bp, Artificial sequence
  Synthetic antisense oligomer
ggtgcccgaagatacagttttcgaactaaa

SEQ ID NO: 29 - DNA, 30 bp, Artificial sequence
  Synthetic antisense oligomer
tggtgcccgaagatacagttttcgaactaa

SEQ ID NO: 30 - DNA, 30 bp, Artificial sequence
  Synthetic antisense oligomer
aaaccttcttctctgtacttaattcaactg

SEQ ID NO: 31 - DNA, 30 bp, Artificial sequence
  Synthetic antisense oligomer
caaaccttcttctctgtacttaattcaact

SEQ ID NO: 32 - DNA, 28 bp, Artificial sequence
  Synthetic antisense oligomer
acaaaccttcttctctgtacttaattca

SEQ ID NO: 33 - DNA, 30 bp, Artificial sequence
  Synthetic antisense oligomer
aacaaaccttcttctctgtacttaattcaa

SEQ ID NO: 34 - DNA, 30 bp, Artificial sequence
  Synthetic antisense oligomer
aaacaaaccttcttctctgtacttaattca

SEQ ID NO: 35 - DNA, 25 bp, Artificial sequence
  Synthetic antisense oligomer
cctcttacctcagttacaatttata

SEQ ID NO: 36 - DNA, 28 bp, Artificial sequence
  Synthetic antisense oligomer
acaaaccttcttctctgtacttaattca

SEQ ID NO: 37 - DNA, 39 bp, Artificial sequence
  Synthetic DNA oligomer
cggtttgtttgggtttgggtttgggtttgggtttgggtt

SEQ ID NO: 38 - DNA, 39 bp, Artificial sequence
  Synthetic DNA oligomer
ggcttgccttacccttacccttacccttacccttaccct

SEQ ID NO: 39 - DNA, 23 bp, Artificial sequence
  Synthetic DNA oligomer
cagcaagtgggaaggtgtaatcc

SEQ ID NO: 40 - DNA, 25 bp, Artificial sequence
  Synthetic DNA oligomer
cccattctatcatcaacgggtacaa

SEQ ID NO: 41 - DNA, 28 bp, Homo sapiens
tgaattaagtacagagaagaaggtttgt